European Patent Application EP 4 707 306 A2, published March 11, 2026. Title: ANTIBODIES TO PLASMINOGEN ACTIVATOR INHIBITOR-1 (PAI-1) AND USES THEREOF. Applicant: SANOFI. The sequence listing filed with the application follows.

SEQUENCE LISTING (170 sequences)

SEQ ID NO: 1 - protein, 379 aa, Homo sapiens [sequence omitted]

SEQ ID NO: 2 - protein, 124 aa, synthetic construct
  REGION 1..124: note = mA105 VH
QVQLQQSGAELMKPGASVKISCKATGFTFSIYWIEWVKQRPGLGLEWIGEILPGSGSTNYNEKFKGKATFTADTSSNTAFMQLSSLTSEDSAVYYCARGGLYYDLDYWGQGTILTVSSAKTTPP

SEQ ID NO: 3 - protein, 115 aa, synthetic construct
  REGION 1..115: note = mA105 VL
DVVMTQTPLTLSVTIGQPASISCKSSQSLLDSDGKTYLNWLLQRPGQSPQRLISLVSKLDSGVPDRFTGSGSGTDFTLKLSRVEGADLGVYYCWQDRHFPRTFGGGTKLEIKRAD

SEQ ID NO: 4 - protein, 125 aa, synthetic construct
  REGION 1..125: note = mA39 VH
QVQLQQSGAELMKPGASVKISCKATGYTFNIYWIQWVKQRPGHGLEWIGEILPGSNTNYNEKFKDKATFTADSSSNTAYMQLSSLTSEDSAVYYCARLGIGLRGALDYWGQGTSVTVSSAKTTPP

SEQ ID NO: 5 - protein, 110 aa, synthetic construct
  REGION 1..110: note = mA39 VL
DIQMTHSPASLSASVGETVTITCRASENIYSYLAWYHQKQGKSPQLLVYNAKTLAEGVPSRFSGSGSGTQFSLNIKSLQPEDFGTFYCQHRYGSPWTFGGGTKLEIKRAD

SEQ ID NO: 6 - protein, 125 aa, synthetic construct
  REGION 1..125: note = mA44 VH
EMQLQESGPSLVKPSQTLSLTCSVTGDSMTNGYWNWIRKFPGNKLEYMGYITYSGSTYYNPSLKGRISITRNTSKNQYYLQLSSVTTEDTATYYCARWHYGSPYYFDYWGQGTTLTVSSAKTTPP

SEQ ID NO: 7 - protein, 110 aa, synthetic construct
  REGION 1..110: note = mA44 VL
DIKMTQSPSSMYASLGERVTITCKASQDINSYLSWLQQKPGKSPKTLIYRANRSVDGVPSRFSGSGSGQDYSLTISSLEYEDMGIYYCLQYDEFPPTFGGGTKLEIKRAD

SEQ ID NO: 8 - protein, 124 aa, synthetic construct
  REGION 1..124: note = mA71 VH
QVQLQQSGAELMKPGASVKISCKATGFTFSTYWIEWIKQRPGHGLDWIGEILPGSGNTNYNEKFKGKATFTADTSSNTVYMQLSSLTSEDSAVYYCARGGLYYNLDSWGQGTTLTVSSAKTTPP

SEQ ID NO: 9 - protein, 115 aa, synthetic construct
  REGION 1..115: note = mA71 VL
DVVMTQTPLTLSVTIGQPASISCKSSQSLLDSDGKTYLYWLLQRPGQSPKRLIYLVSKLDSGVPDRFTGSGSGTDFTLKISRVEAEDLGVYYCWQDTHFPRTFGGGTKLEIKRAD

SEQ ID NO: 10 - protein, 140 aa, synthetic construct
  REGION 1..140: note = mB109 VH
EVQLQQSGSVLARPGTSVKMSCKASGYSFTSYWMHWVKQRPGQGLEWMGAIYPGNSGQGLDWIGAIYPGNSDTTYNQKFEDKAKLTAVASASTAYMEVSSLTNEDSAVYYCTRGLRRWGAMDYWGQGTSVTVSSAKTTPP

SEQ ID NO: 11 - protein, 110 aa, synthetic construct
  REGION 1..110: note = mB109 VL
DIVMTQSHKFMSTSAGDRVSIPCKASQDVSSAVAWYQQKLGQSPKLLIYSASFRYTGVPDRFTGSGSGTDFTFTISSVQAEDLAVYYCQQHYSSPYTFGGGTNLEIKRAD

SEQ ID NO: 12 - protein, 125 aa, synthetic construct
  REGION 1..125: note = mB28 VH
QVQLQQSGAELMKPGASVKISCKATGYTFSISWIEWIKQRPGGLEWIGKILPGSGGANYNEKFKGKATVTADTSSNTVYMQLSSLTSEDSAVYYCARLSTGTRGAFDYWGQGTTLTVSSAKTTPP

SEQ ID NO: 13 - protein, 110 aa, synthetic construct
  REGION 1..110: note = mB28 VL
DIQLTQSPASLSASVGATVTITCRASENVYSYLAWYQQKQGKSPQLLVYNAKTLAEGVPSRFSGSGSGTQFSLKINYLQPEDFGSYYCQHHYGTPPTFGGGTKVEIKRAD

SEQ ID NO: 14 - protein, 121 aa, synthetic construct
  REGION 1..121: note = mC45 VH
QVQLQQSGVELVRPGTSVKVSCKASGYAFTNYLIEWIKQRPGQGLEWIGVIHPGSGVTNYNEKFKGKAILTADKSSSTAYMQLSSLTSDDSAVYFCARDYYGSSHGLMDYWGQGTSVTVSS

SEQ ID NO: 15 - protein, 107 aa, synthetic construct
  REGION 1..107: note = mC45 VL
DIKMTQSPSSMYASLGERVTITCKASQDINSYLSWFQQKPGKSPKTLIYRANRLVDGVPSRFSGSGSGQDYSLTISSLEYEDMGIYYCLQYDEFPRTFGGGTKLEIK

SEQ ID NO: 16 - protein, 118 aa, synthetic construct
  REGION 1..118: note = mE16 VH
EVKLVESGGGLVKPGGSLKLSCAASGFTFSNYGMSWVRQTPEKGLGWVASLRTGGNTYYSDSVKGRFTISRDNDRNILYLQMSSLTSEDTAVYYCARGLRHWGYFDVWGAGTTVTVSS

SEQ ID NO: 17 - protein, 107 aa, synthetic construct
  REGION 1..107: note = mE16 VL
DIVMTQSHKFMSTSVGDRVNITCKASQDVSTAVGWYQQEPGQSPKLLIYSASNRHTGVPDRFTGSGSGTDFTFTISSVQAEDLAVYYCQQHYSSPWTFGGGTKLEIK

SEQ ID NO: 18 - protein, 118 aa, synthetic construct
  REGION 1..118: note = mE21 VH
EVQLQQSGAELVRSGASVKLSCTASGFNIKDYYMHWVKQRPEQGLEWIGWIDPENGDTEYDPKFQAKATMTADTSSNTAYLQLSSLTSEDTAVYYCMYGNYPYYFDYWGQGTTLTVSS

SEQ ID NO: 19 - protein, 107 aa, synthetic construct
  REGION 1..107: note = mE21 VL
DIQMTQTTSSLSASLGDRVTISCRASQDISNYLNWYQQKPDGTVKLLIYYTSRLHSGVPSRFSGSGSGTDYSLTISNLEQEDIATYFCQQGNTLPWTFGGGTKLEIK

SEQ ID NO: 20 - protein, 11 aa, synthetic construct
  REGION 1..11: note = mA105 HCDR3
ARGGLYYDLDY

SEQ ID NO: 21 - protein, 8 aa, synthetic construct
  REGION 1..8: note = mA105 HCDR2
ILPGSGST

SEQ ID NO: 22 - protein, 8 aa, synthetic construct
  REGION 1..8: note = mA105 HCDR1
GFTFSIYW

SEQ ID NO: 23 - protein, 9 aa, synthetic construct
  REGION 1..9: note = mA105 LCDR3
WQDRHFPRT

SEQ ID NO: 24 - skipped

SEQ ID NO: 25 - protein, 11 aa, synthetic construct
  REGION 1..11: note = mA105 LCDR1
QSLLDSDGKTY

SEQ ID NO: 26 - protein, 13 aa, synthetic construct
  REGION 1..13: note = mA39 HCDR3
ARLGIGLRGALDY

SEQ ID NO: 27 - protein, 7 aa, synthetic construct
  REGION 1..7: note = mA39 HCDR2
ILPGSNT

SEQ ID NO: 28 - protein, 8 aa, synthetic construct
  REGION 1..8: note = mA39 HCDR1
GYTFNIYW

SEQ ID NO: 29 - protein, 9 aa, synthetic construct
  REGION 1..9: note = mA39 LCDR3
QHRYGSPWT

SEQ ID NO: 30 - skipped

SEQ ID NO: 31 - protein, 6 aa, synthetic construct
  REGION 1..6: note = mA38 LCDR1
ENIYSY

SEQ ID NO: 32 - protein, 13 aa, synthetic construct
  REGION 1..13: note = mA44 HCDR3
ARWHYGSPYYFDY

SEQ ID NO: 33 - protein, 7 aa, synthetic construct
  REGION 1..7: note = mA44 HCDR2
ITYSGST

SEQ ID NO: 34 - protein, 8 aa, synthetic construct
  REGION 1..8: note = mA44 HCDR1
GDSMTNGY

SEQ ID NO: 35 - protein, 9 aa, synthetic construct
  REGION 1..9: note = mA44 LCDR3
LQYDEFPPT

SEQ ID NO: 36 - skipped

SEQ ID NO: 37 - protein, 6 aa, synthetic construct
  REGION 1..6: note = mA44 LCDR1
QDINSY

SEQ ID NO: 38 - protein, 11 aa, synthetic construct
  REGION 1..11: note = mA71 HCDR3
ARGGLYYNLDS

SEQ ID NO: 39 - protein, 8 aa, synthetic construct
  REGION 1..8: note = mA71 HCDR2
ILPGSGNT

SEQ ID NO: 40 - protein, 8 aa, synthetic construct
  REGION 1..8: note = mA71 HCDR1
GFTFSTYW

SEQ ID NO: 41 - protein, 9 aa, synthetic construct
  REGION 1..9: note = mA71 LCDR3
WQDTHFPRT

SEQ ID NO: 42 - skipped

SEQ ID NO: 43 - protein, 11 aa, synthetic construct
  REGION 1..11: note = mA71 LCDR1
QSLLDSDGKTY

SEQ ID NO: 44 - protein, 11 aa, synthetic construct
  REGION 1..11: note = mA75 HCDR3
ARGGLYYAMDY

SEQ ID NO: 45 - protein, 8 aa, synthetic construct
  REGION 1..8: note = mA75 HCDR2
ILPGSGLT

SEQ ID NO: 46 - protein, 8 aa, synthetic construct
  REGION 1..8: note = mA75 HCDR1
GFTFSTYW

SEQ ID NO: 47 - protein, 9 aa, synthetic construct
  REGION 1..9: note = mA75 LCDR3
WQGSHFPQT

SEQ ID NO: 48 - skipped

SEQ ID NO: 49 - protein, 11 aa, synthetic construct
  REGION 1..11: note = mA75 LCDR1
QSLLDSEGKTY

SEQ ID NO: 50 - protein, 12 aa, synthetic construct
  REGION 1..12: note = mB109 HCDR3
TRGLRRWGAMDY

SEQ ID NO: 51 - protein, 8 aa, synthetic construct
  REGION 1..8: note = mB109 HCDR2
ILPGSGLT

SEQ ID NO: 52 - protein, 8 aa, synthetic construct
  REGION 1..8: note = mB109 HCDR1
GFTFSTYW

SEQ ID NO: 53 - protein, 9 aa, synthetic construct
  REGION 1..9: note = mB109 LCDR3
QQHYSSPYT

SEQ ID NO: 54 - skipped

SEQ ID NO: 55 - protein, 6 aa, synthetic construct
  REGION 1..6: note = mB109 LCDR1
QDVSSA

SEQ ID NO: 56 - protein, 13 aa, synthetic construct
  REGION 1..13: note = mB28 HCDR3
ARLSTGTRGAFDY

SEQ ID NO: 57 - protein, 8 aa, synthetic construct
  REGION 1..8: note = mB28 HCDR2
ILPGSGGA

SEQ ID NO: 58 - protein, 8 aa, synthetic construct
  REGION 1..8: note = mB28 HCDR1
GYTFSISW

SEQ ID NO: 59 - protein, 9 aa, synthetic construct
  REGION 1..9: note = mB28 LCDR3
QHHYGTPPT

SEQ ID NO: 60 - skipped

SEQ ID NO: 61 - protein, 6 aa, synthetic construct
  REGION 1..6: note = mB28 LCDR1
ENVYSY

SEQ ID NO: 62 - protein, 14 aa, synthetic construct
  REGION 1..14: note = mC45 HCDR3
ARDYYGSSHGLMDY

SEQ ID NO: 63 - protein, 8 aa, synthetic construct
  REGION 1..8: note = mC45 HCDR2
IHPGSGVT

SEQ ID NO: 64 - protein, 8 aa, synthetic construct
  REGION 1..8: note = mC45 HCDR1
GYAFTNYL

SEQ ID NO: 65 - protein, 9 aa, synthetic construct
  REGION 1..9: note = mC45 LCDR3
LQYDEFPRT

SEQ ID NO: 66 - skipped

SEQ ID NO: 67 - protein, 6 aa, synthetic construct
  REGION 1..6: note = mC45 LCDR1
QDINSY

SEQ ID NO: 68 - protein, 12 aa, synthetic construct
  REGION 1..12: note = mE16 HCDR3
ARGLRHWGYFDV

SEQ ID NO: 69 - protein, 7 aa, synthetic construct
  REGION 1..7: note = mE16 HCDR2
LRTGGNT

SEQ ID NO: 70 - protein, 8 aa, synthetic construct
  REGION 1..8: note = mE16 HCDR1
GFTFSNYG

SEQ ID NO: 71 - protein, 9 aa, synthetic construct
  REGION 1..9: note = mE16 LCDR3
QQHYSSPWT

SEQ ID NO: 72 - skipped

SEQ ID NO: 73 - protein, 6 aa, synthetic construct
  REGION 1..6: note = mE16 LCDR1
QDISNY

SEQ ID NO: 74 - protein, 11 aa, synthetic construct
  REGION 1..11: note = mE21 HCDR3
MYGNYPYYFDY

SEQ ID NO: 75 - protein, 8 aa, synthetic construct
  REGION 1..8: note = mE21 HCDR2
IDPENGDT

SEQ ID NO: 76 - protein, 8 aa, synthetic construct
  REGION 1..8: note = mE21 HCDR1
GFNIKDYY

SEQ ID NO: 77 - protein, 9 aa, synthetic construct
  REGION 1..9: note = mE21 LCDR3
QQGNTLPWT

SEQ ID NO: 78 - skipped

SEQ ID NO: 79 - protein, 6 aa, synthetic construct
  REGION 1..6: note = mE21 LCDR1
QDISNY

SEQ ID NO: 80 - protein, 124 aa, synthetic construct
  REGION 1..124: note = mA75 VH
QGQLQQSGAELMKPGASVKISCKASGFTFSTYWIAWLKQRPGHGLEWIAEILPGSGLTNYNEIFRGKATFTADTSSNTAYMQLSSLTSEDSAVYYCARGGLYYAMDYWGQGTSVTVSSAKTTAP

SEQ ID NO: 81 - protein, 114 aa, synthetic construct
  REGION 1..114: note = mA75 VL
DVVMTQTPLTLSVTIGQPASICKSSQSLLDSEGKTYLNWLFQRPGQSPKRLIYLVCKLDCGVPDRFTGSGSGTDFTLKISRVEGEDLGVYYCWQGSHFPQTFGGGTKLEIKRAD

SEQ ID NO: 82 - protein, 119 aa, synthetic construct
  REGION 1..119: note = HC1a
EMTLKESGPTLVKPTQTLSLTCSVTGDSMTNGYWNWIRKFPGKALEYMGYITYSGSTYYNPSLKGRISITRNTSKNQYYLTLSSVTTVDTATYYCARWHYGSPYYFDYWGQGTTLTVSS

SEQ ID NO: 83 - protein, 119 aa, synthetic construct
  REGION 1..119: note = HC1b
EMQLQESGPGLVKPSETLSLTCSVTGDSMTNGYWNWIRKFPGKGLEYMGYITYSGSTYYNPSLKGRISITRNTSKNQYYLKLSSVTTADTATYYCARWHYGSPYYFDYWGQGTTLTVSS

SEQ ID NO: 84 - protein, 119 aa, synthetic construct
  REGION 1..119: note = HC2a
EMTLKESGPTLVKPTQTLSLTCSVTGESMTQGYWNWIRKFPGKALEYMGYITYSGSTYYNPSLKGRISITRQTSKNQYYLTLSSVTTVETATYYCARWHYGSPYYFDYWGQGTTLTVSS

SEQ ID NO: 85 - protein, 119 aa, synthetic construct
  REGION 1..119: note = HC2b
EMTLKESGPTLVKPTQTLSLTCSVTGDSMTQGYWNWIRKFPGKALEYMGYITYSGSTYYNPSLKGRISITRNTSKNQYYLTLSSVTTVDTATYYCARWHYGSPYYFDYWGQGTTLTVSS

SEQ ID NO: 86 - protein, 119 aa, synthetic construct
  REGION 1..119: note = HC3
QMTLKESGPTLVKPTQTLSLTCSVSGDSMTNGYWNWIRQFPGKALEYMGYITYSGSTYYNPSLKGRITITRDTSKNQYYLTLSSVTTVDTATYYCARWHYGSPYYFDYWGQGTTLTVSS

SEQ ID NO: 87 - protein, 119 aa, synthetic construct
  REGION 1..119: note = HC4
QMTLKESGPTLVKPTQTLSLTCSVSGESMTQGYWNWIRQFPGKALEYMGYITYSGSTYYNPSLKGRITITRQTSKNQYYLTLSSVTTVETATYYCARWHYGSPYYFDYWGQGTTLTVSS

SEQ ID NO: 88 - protein, 119 aa, synthetic construct
  REGION 1..119: note = HC5a
QVQLQESGPGLVKPSETLSLTCTVSGDSMTNGYWNWIRQPPGKGLEYMGYITYSGSTYYNPSLKSRITISRNTSKNQYSLKLSSVTAADTAVYYCARWHYGSPYYFDYWGQGTLVTVSS

SEQ ID NO: 89 - protein, 119 aa, synthetic construct
  REGION 1..119: note = HC5b
QMQLQESGPGLVKPSETLSLTCTVSGDSMTNGYWNWIRQPPGKGLEYMGYITYSGSTYYNPSLKSRITISRDTSKNQYSLKLSSVTAADTAVYYCARWHYGSPYYFDYWGQGTLVTVSS

SEQ ID NO: 90 - protein, 119 aa, synthetic construct
  REGION 1..119: note = HC5c
QMQLQQSGPGLVKPSQTLSLTCAISGDSMTNGYWNWIRQSPSRGLEYMGYITYSGSTYYAVSVKSRITINRDTSKNQYSLQLSSVTPEDTAVYYCARWHYGSPYYFDYWGQGTLVTVSS

SEQ ID NO: 91 - protein, 107 aa, synthetic construct
  REGION 1..107: note = LC1a
DIKMTQSPSSLSASVGDRVTITCKASQDINSYLSWLQQKPGKSPKTLIYRANRSVDGVPSRFSGSGSGQDYSLTISSLQPEDLGIYYCLQYDEFPPTFGGGTKLEIK

SEQ ID NO: 92 - protein, 107 aa, synthetic construct
  REGION 1..107: note = LC1b
DIKMTQSPSSVSVSPGQTVTITCKASQDINSYLSWLQQKPGQSPKTLIYRANRSVDGVPSRFSGSGSGQDYSLTISSLQAMDEGIYYCLQYDEFPPTFGGGTKLTIK

SEQ ID NO: 93 - protein, 107 aa, synthetic construct
  REGION 1..107: note = LC2
DIKMTQSPSSLSASVGDRVTITCKASQDINSYLSWLQQKPGKSPKTLIYRAQRSVEGVPSRFSGSGSGQDYSLTISSLQPEDLGIYYCLQYDEFPPTFGGGTKLEIK

SEQ ID NO: 94 - protein, 107 aa, synthetic construct
  REGION 1..107: note = LC3
DIKMTQSPSSLSASVGDRVTITCKASQDINSYLSWLQQKPGKSPKTLIYRANRSVDGVPSRFSGSGSGQDYSLTISSLQPEDLATYYCLQYDEFPPTFGGGTKLEIK

SEQ ID NO: 95 - protein, 107 aa, synthetic construct
  REGION 1..107: note = LC4
DIKMTQSPSSLSASVGDRVTITCKASQDINSYLSWLQQKPGKSPKTLIYRAQRSVEGVPSRFSGSGSGQDYSLTISSLQPEDLATYYCLQYDEFPPTFGGGTKLEIK

SEQ ID NO: 96 - protein, 107 aa, synthetic construct
  REGION 1..107: note = LC5a
DIQMTQSPSSLSASVGDRVTITCKASQDINSYLSWLQQKPGKAPKLLIYRANRSVDGVPSRFSGSGSGTDYTFTISSLQPEDIATYYCLQYDEFPPTFGGGTKVEIK

SEQ ID NO: 97 - protein, 107 aa, synthetic construct
  REGION 1..107: note = LC5b
DIQMTQSPSSLSASVGDRVTITCKASQDINSYLSWLQQKPGKAPKTLIYRANRSVDGVPSRFSGSGSGQDYTFTISSLQPEDIATYYCLQYDEFPPTFGGGTKVEIK

SEQ ID NO: 98 - protein, 107 aa, synthetic construct
  REGION 1..107: note = LC5c
EIVMTQSPATLSLSPGERATLSCKASQDINSYLSWLQQKPGQAPRTLIYRANRSVDGIPARFSGSGSGQDYTLTISSLEPEDFAVYYCLQYDEFPPTFGGGTKVEIK

SEQ ID NO: 99 - protein, 255 aa, synthetic construct
  REGION 1..255: note = CH
ASTKGPSVFPLAPSSKSTSGGTAALGCLVKDYFPEPVTVSWNSGALTSGVHTFPAVLQSSGLYSLSSVVTVPSSSLGTQTYICNVNHKPSNTKVDKKVEPKSCDKTHTCPPCPAPELLGGPSVFLFPPKPKDTLMISRTPEVTCVVVDVSHEDPEVKFNWYVDGVEVHNAKTKPREEQYNSTYRVVSVLTVLHQDWLNGKEYKCKVSNKALPAPIEKTISKAKGQPREPQVYTLPPSRDELTKNQVSLTCLVKGF

SEQ ID NO: 100 - protein, 107 aa, synthetic construct [sequence omitted]

SEQ ID NO: 101 - protein, 107 aa, synthetic construct
  REGION 1..107: note = vk1
DIQMTQSPSSLSASVGDRVTITCRASQSISSYLNWYQQKPGKAPKLLIYAASSLQSGVPSRFSGSGSGTDFTLTISSLQPEDLATYYCQQSYSTPPTFGQGTKVEIK

SEQ ID NO: 102 - protein, 106 aa, synthetic construct
  REGION 1..106: note = vlambda3
  SITE 22: note = misc_feature - X can be any naturally occurring amino acid
  SITE 87: note = misc_feature - X can be any naturally occurring amino acid
SYELTQPPSVSVSPGQTASITXSGDKLGDKYASWYQQKPGQSPVLVIYQDSKRPSGIPERFSGSNSGNTATLTISGTQAMDEADYYXQAWDSSAVVFGGGTKLTVL

SEQ ID NO: 103 - protein, 120 aa, synthetic construct
  REGION 1..120: note = vh2
QVTLKESGPTLVKPTQTLTLTCTFSGFSLSTSGVGVGWIRQPPGKALEWLARIDWDDDKYYSTSLKTRLTISKDTSKNQVVLTMTNMDPVDTATYYCARMGFTGTYFDYWGQGTLVTVSS

SEQ ID NO: 104 - protein, 118 aa, synthetic construct
  REGION 1..118: note = vh4
  SITE 22: note = misc_feature - X can be any naturally occurring amino acid
  SITE 95: note = misc_feature - X can be any naturally occurring amino acid
QVQLQESGPGLVKPSETLSLTXTVSGGSISSYYWSWIRQPPGKGLEWIGYIYYSGSTNYNPSLKSRVTISVDTSKNQFSLKLSSVTAADTAVYYXARGDSSGYYFDYWGQGTLVTVSS

SEQ ID NO: 105 - DNA, 21 bp, synthetic construct
  misc_feature 1..21: note = Heavy Chain 3'- Primer
  source 1..21: mol_type = other DNA
tatgcaaggcttacaaccaca

SEQ ID NO: 106 - DNA, 24 bp, synthetic construct
  misc_feature 1..24: note = Light Chain 3'- Primer
  source 1..24: mol_type = other DNA
ctcattcctgttgaagctcttgag

SEQ ID NO: 107 - protein, 107 aa, synthetic construct
  REGION 1..107: note = IGKV1-33-01_IGKJ4-01
DIQMTQSPSSLSASVGDRVTITCQASQDISNYLNWYQQKPGKAPKLLIYDASNLETGVPSRFSGSGSGTDFTFTISSLQPEDIATYYCQQYDNLPLTFGGGTKVEIK

SEQ ID NO: 108 - protein, 119 aa, synthetic construct
  REGION 1..119: note = IGHV4-59-02_IGHD6-13-01_IGHJ4-02
QVQLQESGPGLVKPSETLSLTCTVSGGSVSSYYWSWIRQPPGKGLEWIGYIYYSGSTNYNPSLKSRVTISVDTSKNQFSLKLSSVTAADTAVYYCARGYSSSWYYFDYWGQGTLVTVSS

SEQ ID NO: 109 - protein, 226 aa, synthetic construct
  REGION 1..226: note = A44-hv1LC1a x HC1a
DIKMTQSPSSLSASVGDRVTITCKASQDINSYLSWLQQKPGKSPKTLIYRANRSVDGVPSRFSGSGSGQDYSLTISSLQPEDLGIYYCLQYDEFPPTFGGGTKLEIKEMTLKESGPTLVKPTQTLSLTCSVTGDSMTNGYWNWIRKFPGKALEYMGYITYSGSTYYNPSLKGRISITRNTSKNQYYLTLSSVTTVDTATYYCARWHYGSPYYFDYWGQGTTLTVSS

SEQ ID NO: 110 - protein, 226 aa, synthetic construct
  REGION 1..226: note = A44-hv2LC1b x HC1b
DIKMTQSPSSVSVSPGQTVTITCKASQDINSYLSWLQQKPGQSPKTLIYRANRSVDGVPSRFSGSGSGQDYSLTISSLQAMDEGIYYCLQYDEFPPTFGGGTKLTIKEMQLQESGPGLVKPSETLSLTCSVTGDSMTNGYWNWIRKFPGKGLEYMGYITYSGSTYYNPSLKGRISITRNTSKNQYYLKLSSVTTADTATYYCARWHYGSPYYFDYWGQGTTLTVSS

SEQ ID NO: 111 - protein, 226 aa, synthetic construct
  REGION 1..226: note = A44-hv3LC2 x HC2a
DIKMTQSPSSLSASVGDRVTITCKASQDINSYLSWLQQKPGKSPKTLIYRAQRSVEGVPSRFSGSGSGQDYSLTISSLQPEDLGIYYCLQYDEFPPTFGGGTKLEIKEMTLKESGPTLVKPTQTLSLTCSVTGESMTQGYWNWIRKFPGKALEYMGYITYSGSTYYNPSLKGRISITRQTSKNQYYLTLSSVTTVETATYYCARWHYGSPYYFDYWGQGTTLTVSS

SEQ ID NO: 112 - protein, 226 aa, synthetic construct
  REGION 1..226: note = A44-hv4LC1a x HC2b
DIKMTQSPSSLSASVGDRVTITCKASQDINSYLSWLQQKPGKSPKTLIYRANRSVDGVPSRFSGSGSGQDYSLTISSLQPEDLGIYYCLQYDEFPPTFGGGTKLEIKEMTLKESGPTLVKPTQTLSLTCSVTGDSMTQGYWNWIRKFPGKALEYMGYITYSGSTYYNPSLKGRISITRNTSKNQYYLTLSSVTTVDTATYYCARWHYGSPYYFDYWGQGTTLTVSS

SEQ ID NO: 113 - protein, 226 aa, synthetic construct
  REGION 1..226: note = A44-hv5LC2 x HC2b
DIKMTQSPSSLSASVGDRVTITCKASQDINSYLSWLQQKPGKSPKTLIYRAQRSVEGVPSRFSGSGSGQDYSLTISSLQPEDLGIYYCLQYDEFPPTFGGGTKLEIKEMTLKESGPTLVKPTQTLSLTCSVTGDSMTQGYWNWIRKFPGKALEYMGYITYSGSTYYNPSLKGRISITRNTSKNQYYLTLSSVTTVDTATYYCARWHYGSPYYFDYWGQGTTLTVSS

SEQ ID NO: 114 - protein, 226 aa, synthetic construct
  REGION 1..226: note = A44-hv6LC3 x HC3
DIKMTQSPSSLSASVGDRVTITCKASQDINSYLSWLQQKPGKSPKTLIYRANRSVDGVPSRFSGSGSGQDYSLTISSLQPEDLATYYCLQYDEFPPTFGGGTKLEIKQMTLKESGPTLVKPTQTLSLTCSVSGDSMTNGYWNWIRQFPGKALEYMGYITYSGSTYYNPSLKGRITITRDTSKNQYYLTLSSVTTVDTATYYCARWHYGSPYYFDYWGQGTTLTVSS

SEQ ID NO: 115 - protein, 226 aa, synthetic construct
  REGION 1..226: note = A44-hv7LC4 x HC4
DIKMTQSPSSLSASVGDRVTITCKASQDINSYLSWLQQKPGKSPKTLIYRAQRSVEGVPSRFSGSGSGQDYSLTISSLQPEDLATYYCLQYDEFPPTFGGGTKLEIKQMTLKESGPTLVKPTQTLSLTCSVSGESMTQGYWNWIRQFPGKALEYMGYITYSGSTYYNPSLKGRITITRQTSKNQYYLTLSSVTTVETATYYCARWHYGSPYYFDYWGQGTTLTVSS

SEQ ID NO: 116 - protein, 226 aa, synthetic construct
  REGION 1..226: note = A44-hv8LC5a x HC5a
DIQMTQSPSSLSASVGDRVTITCKASQDINSYLSWLQQKPGKAPKLLIYRANRSVDGVPSRFSGSGSGTDYTFTISSLQPEDIATYYCLQYDEFPPTFGGGTKVEIKQVQLQESGPGLVKPSETLSLTCTVSGDSMTNGYWNWIRQPPGKGLEYMGYITYSGSTYYNPSLKSRITISRNTSKNQYSLKLSSVTAADTAVYYCARWHYGSPYYFDYWGQGTLVTVSS

SEQ ID NO: 117 - protein, 226 aa, synthetic construct
  REGION 1..226: note = A44-hv9LC5b x HC5b
DIQMTQSPSSLSASVGDRVTITCKASQDINSYLSWLQQKPGKAPKTLIYRANRSVDGVPSRFSGSGSGQDYTFTISSLQPEDIATYYCLQYDEFPPTFGGGTKVEIKQMQLQESGPGLVKPSETLSLTCTVSGDSMTNGYWNWIRQPPGKGLEYMGYITYSGSTYYNPSLKSRITISRDTSKNQYSLKLSSVTAADTAVYYCARWHYGSPYYFDYWGQGTLVTVSS

SEQ ID NO: 118 - protein, 226 aa, synthetic construct
  REGION 1..226: note = A44-hv10LC5c x HC5c
EIVMTQSPATLSLSPGERATLSCKASQDINSYLSWLQQKPGQAPRTLIYRANRSVDGIPARFSGSGSGQDYTLTISSLEPEDFAVYYCLQYDEFPPTFGGGTKVEIKQMQLQQSGPGLVKPSQTLSLTCAISGDSMTNGYWNWIRQSPSRGLEYMGYITYSGSTYYAVSVKSRITINRDTSKNQYSLQLSSVTPEDTAVYYCARWHYGSPYYFDYWGQGTLVTVSS

SEQ ID NO: 119 - protein, 226 aa, synthetic construct
  REGION 1..226: note = A44-hv11LC2 x HC3
DIKMTQSPSSLSASVGDRVTITCKASQDINSYLSWLQQKPGKSPKTLIYRAQRSVEGVPSRFSGSGSGQDYSLTISSLQPEDLGIYYCLQYDEFPPTFGGGTKLEIKQMTLKESGPTLVKPTQTLSLTCSVSGDSMTNGYWNWIRQFPGKALEYMGYITYSGSTYYNPSLKGRITITRDTSKNQYYLTLSSVTTVDTATYYCARWHYGSPYYFDYWGQGTTLTVSS

SEQ ID NO: 120 - protein, 226 aa, synthetic construct
  REGION 1..226: note = A44-hv12LC4 X HC3
DIKMTQSPSSLSASVGDRVTITCKASQDINSYLSWLQQKPGKSPKTLIYRAQRSVEGVPSRFSGSGSGQDYSLTISSLQPEDLATYYCLQYDEFPPTFGGGTKLEIKQMTLKESGPTLVKPTQTLSLTCSVSGDSMTNGYWNWIRQFPGKALEYMGYITYSGSTYYNPSLKGRITITRDTSKNQYYLTLSSVTTVDTATYYCARWHYGSPYYFDYWGQGTTLTVSS

SEQ ID NO: 121 - protein, 226 aa, synthetic construct
  REGION 1..226: note = A44-hv13LC2 x HC5b
DIKMTQSPSSLSASVGDRVTITCKASQDINSYLSWLQQKPGKSPKTLIYRAQRSVEGVPSRFSGSGSGQDYSLTISSLQPEDLGIYYCLQYDEFPPTFGGGTKLEIKQMQLQESGPGLVKPSETLSLTCTVSGDSMTNGYWNWIRQPPGKGLEYMGYITYSGSTYYNPSLKSRITISRDTSKNQYSLKLSSVTAADTAVYYCARWHYGSPYYFDYWGQGTLVTVSS

SEQ ID NO: 122 - protein, 226 aa, synthetic construct
  REGION 1..226: note = A44-hv14LC4 x HC5b
DIKMTQSPSSLSASVGDRVTITCKASQDINSYLSWLQQKPGKSPKTLIYRAQRSVEGVPSRFSGSGSGQDYSLTISSLQPEDLATYYCLQYDEFPPTFGGGTKLEIKQMQLQESGPGLVKPSETLSLTCTVSGDSMTNGYWNWIRQPPGKGLEYMGYITYSGSTYYNPSLKSRITISRDTSKNQYSLKLSSVTAADTAVYYCARWHYGSPYYFDYWGQGTLVTVSS

SEQ ID NO: 123 - DNA, 255 bp, synthetic construct
  misc_feature 1..255: note = HC1a
  source 1..255: mol_type = other DNA
gagatgaccctgaaagagtccggccccaccctggtcaaacccacccagaccctgagcctgacctgcagcgtgaccggcgacagcatgaccaacggctactggaactggatccggaagttccccggcaaggccctcgagtacatgggctacatcacctacagcggcagcacctactacaaccccagcctgaagggccggatcagcatcacccggaacaccagcaagaaccagtactacctgaccctgtccagcgtg

SEQ ID NO: 124 - DNA, 255 bp, synthetic construct
  misc_feature 1..255: note = HC1b
  source 1..255: mol_type = other DNA
gagatgcagctgcaggaaagcggccctggcctggtcaaacccagcgagacactgagcctgacctgcagcgtgaccggcgacagcatgaccaacggctactggaactggatccggaagttccccggcaagggcctcgagtacatgggctacatcacctacagcggcagcacctactacaaccccagcctgaagggccggatcagcatcacccggaacaccagcaagaaccagtactacctgaagctgtccagcgtg

SEQ ID NO: 125 - DNA, 255 bp, synthetic construct
  misc_feature 1..255: note = HC2a
  source 1..255: mol_type = other DNA
gagatgaccctgaaagagtccggccccaccctggtcaaacccacccagaccctgagcctgacctgcagcgtgaccggcgagagcatgacccagggctactggaactggatccggaagttccccggcaaggccctcgagtacatgggctacatcacctacagcggcagcacctactacaaccccagcctgaagggccggatcagcatcacccggcagaccagcaagaaccagtactacctgaccctgtccagcgtg

SEQ ID NO: 126 - DNA, 255 bp, synthetic construct
  misc_feature 1..255: note = HC2b
  source 1..255: mol_type = other DNA
gagatgaccctgaaagagtccggccccaccctggtcaaacccacccagaccctgagcctgacctgcagcgtgaccggcgacagcatgacccagggctactggaactggatccggaagttccccggcaaggccctcgagtacatgggctacatcacctacagcggcagcacctactacaaccccagcctgaagggccggatcagcatcacccggaacaccagcaagaaccagtactacctgaccctgtccagcgtg

SEQ ID NO: 127 - DNA, 255 bp, synthetic construct
  misc_feature 1..255: note = HC3
  source 1..255: mol_type = other DNA
cagatgaccctgaaagagtccggccccaccctggtcaaacccacccagaccctgagcctgacctgcagcgtgtccggcgacagcatgaccaacggctactggaactggatccggcagttccccggcaaggccctcgagtacatgggctacatcacctacagcggcagcacctactacaaccccagcctgaagggccggatcaccatcacccgggacaccagcaagaaccagtactacctgaccctgagcagcgtg

SEQ ID NO: 128 - DNA, 255 bp, synthetic construct
  misc_feature 1..255: note = HC4
  source 1..255: mol_type = other DNA
cagatgaccctgaaagagtccggccccaccctggtcaaacccacccagaccctgagcctgacctgcagcgtgtccggcgagagcatgacccagggctactggaactggatccggcagttccccggcaaggccctcgagtacatgggctacatcacctacagcggcagcacctactacaaccccagcctgaagggccggatcaccatcacccggcagaccagcaagaaccagtactacctgaccctgagcagcgtg

SEQ ID NO: 129 - DNA, 255 bp, synthetic construct
  misc_feature 1..255: note = HC5a
  source 1..255: mol_type = other DNA
caggtgcagctgcaggaaagcggccctggcctggtcaaacccagcgagacactgagcctgacctgcaccgtgtccggcgacagcatgaccaacggctactggaactggatccggcagccccctggcaagggcctcgagtacatgggctacatcacctacagcggcagcacctactacaaccccagcctgaagtcccggatcaccatcagccggaacaccagcaagaaccagtacagcctgaagctgagcagcgtg

SEQ ID NO: 130 - DNA, 255 bp, synthetic construct
  misc_feature 1..255: note = HC5b
  source 1..255: mol_type = other DNA
cagatgcagctgcaggaaagcggccctggcctggtcaaacccagcgagacactgagcctgacctgcaccgtgtccggcgacagcatgaccaacggctactggaactggatccggcagccccctggcaagggcctcgagtacatgggctacatcacctacagcggcagcacctactacaaccccagcctgaagtcccggatcaccatcagccgggacaccagcaagaaccagtacagcctgaagctgagcagcgtg

SEQ ID NO: 131 - DNA, 255 bp, synthetic construct
  misc_feature 1..255: note = HC5c
  source 1..255: mol_type = other DNA
cagatgcagctgcagcagagcggccctggcctggtcaaacccagccagaccctgagcctgacctgcgccatcagcggcgacagcatgaccaacggctactggaactggatccggcagagccccagcagaggcctcgagtacatgggctacatcacctacagcggcagcacctactacgccgtgtccgtgaagtcccggatcaccatcaaccgggacaccagcaagaaccagtacagcctgcagctgagcagcgtg

SEQ ID NO: 132 - DNA, 255 bp, synthetic construct
  misc_feature 1..255: note = LC1a
  source 1..255: mol_type = other DNA
gacatcaagatgacccagagccccagcagcctgagcgccagcgtgggcgacagagtgaccatcacatgcaaggccagccaggacatcaacagctacctgagctggctgcagcagaagcccggcaagagccccaagaccctgatctaccgggccaaccgcagcgtggacggcgtgccaagcagattttccggcagcggcagcggccaggactacagcctgaccatcagcagcctgcagcccgaggacctgggcatc

SEQ ID NO: 133 - DNA, 255 bp, synthetic construct
  misc_feature 1..255: note = LC1b
  source 1..255: mol_type = other DNA
gacatcaagatgacccagagccccagcagcgtgtccgtgtctcctggccagaccgtgaccatcacatgcaaggccagccaggacatcaacagctacctgagctggctgcagcagaagcccggccagtcccccaagaccctgatctaccgggccaaccgcagcgtggacggcgtgccaagcagattttccggcagcggcagcggccaggactacagcctgaccatcagcagcctgcaggccatggacgagggcatc

SEQ ID NO: 134 - DNA, 255 bp, synthetic construct
  misc_feature 1..255: note = LC2
  source 1..255: mol_type = other DNA
gacatcaagatgacccagagccccagcagcctgagcgccagcgtgggcgacagagtgaccatcacatgcaaggccagccaggacatcaacagctacctgagctggctgcagcagaagcccggcaagagccccaagaccctgatctaccgggcccagcggagcgtggaaggcgtgccaagcagattcagcggcagcggctccggccaggactacagcctgaccatcagcagcctgcagcccgaggacctgggcatc

SEQ ID NO: 135 - DNA, 255 bp, synthetic construct
  misc_feature 1..255: note = LC3
  source 1..255: mol_type = other DNA
gacatcaagatgacccagagccccagcagcctgagcgccagcgtgggcgacagagtgaccatcacatgcaaggccagccaggacatcaacagctacctgagctggctgcagcagaagcccggcaagagccccaagaccctgatctaccgggccaaccgcagcgtggacggcgtgccaagcagattttccggcagcggcagcggccaggactacagcctgaccatcagcagcctgcagcccgaggacctggccacc

SEQ ID NO: 136 - DNA, 255 bp, synthetic construct
  misc_feature 1..255: note = LC4
  source 1..255: mol_type = other DNA
gacatcaagatgacccagagccccagcagcctgagcgccagcgtgggcgacagagtgaccatcacatgcaaggccagccaggacatcaacagctacctgagctggctgcagcagaagcccggcaagagccccaagaccctgatctaccgggcccagcggagcgtggaaggcgtgccaagcagattcagcggcagcggctccggccaggactacagcctgaccatcagcagcctgcagcccgaggacctggccacc

SEQ ID NO: 137 - DNA, 255 bp, synthetic construct
  misc_feature 1..255: note = LC5a
  source 1..255: mol_type = other DNA
gacatccagatgacccagagccccagcagcctgagcgccagcgtgggcgacagagtgaccatcacatgcaaggccagccaggacatcaacagctacctgagctggctgcagcagaagcccggcaaggcccccaagctgctgatctaccgggccaaccgcagcgtggacggcgtgccaagcagattttccggcagcggctccggcaccgactacaccttcaccatcagcagcctgcagcccgaggatatcgccacc

SEQ ID NO: 138 - DNA, 255 bp, synthetic construct
  misc_feature 1..255: note = LC5b
  source 1..255: mol_type = other DNA
gacatccagatgacccagagccccagcagcctgagcgccagcgtgggcgacagagtgaccatcacatgcaaggccagccaggacatcaacagctacctgagctggctgcagcagaagcccggcaaggcccccaagaccctgatctaccgggccaaccgcagcgtggacggcgtgccaagcagattttccggcagcggcagcggccaggactacaccttcaccatcagcagcctgcagcccgaggatatcgccacc

SEQ ID NO: 139 - DNA, 255 bp, synthetic construct
  misc_feature 1..255: note = LC5c
  source 1..255: mol_type = other DNA
gagatcgtgatgacccagagccccgccaccctgtctctgagccctggcgagagagccaccctgagctgcaaggccagccaggacatcaacagctacctgagctggctgcagcagaagcccggccaggcccccagaaccctgatctaccgggccaacagaagcgtggacggcatccccgccagattcagcggcagcggctccggccaggactacaccctgaccatcagcagcctggaacccgaggacttcgccgtg

SEQ ID NO: 140 - protein, 119 aa, synthetic construct
  REGION 1..119: note = mA44 VH
EMQLQESGPSLVKPSQTLSLTCSVTGDSMTNGYWNWIRKFPGNKLEYMGYITYSGSTYYNPSLKGRISITRNTSKNQYYLQLSSVTTEDTATYYCARWHYGSPYYFDYWGQGTTLTVSS

SEQ ID NO: 141 - protein, 107 aa, synthetic construct
  REGION 1..107: note = mA44 VL
DIKMTQSPSSMYASLGERVTITCKASQDINSYLSWLQQKPGKSPKTLIYRANRSVDGVPSRFSGSGSGQDYSLTISSLEYEDMGIYYCLQYDEFPPTFGGGTKLEIK

SEQ ID NO: 142 - protein, 118 aa, synthetic construct
  REGION 1..118: note = mA44 VL
DIKMTQSPSSMYASLGERVTITCKASQDINSYLSWLQQKPGKSPKTLIYRANRSVDGVPSRFSGSGSGQDYSLTISSLEYEDMGIYYCLQYDEFPPTFGGGTKLEIKRADAAPTVSIF

SEQ ID NO: 143 - protein, 107 aa, synthetic construct
  REGION 1..107: note = IGKV3-11-02_IGKJ4-0
EIVLTQSPATLSLSPGERATLSCRASQSVSSYLAWYQQKPGQAPRLLIYDASNRATGIPARFSGSGSGRDFTLTISSLEPEDFAVYYCQQRSNWPLTFGGGTKVEIK

SEQ ID NO: 144 - protein, 123 aa, synthetic construct
  REGION 1..123: note = IGHV6-1-02_IGHD6-13-01_IGHJ4-02
QVQLQQSGPGLVKPSQTLSLTCAISGDSVSSNSAAWNWIRQSPSRGLEWLGRTYYRSKWYNDYAVSVKSRITINPDTSKNQFSLQLNSVTPEDTAVYYCARGYSSSWYYFDYWGQGTLVTVSS

SEQ ID NO: 145 - skipped

SEQ ID NO: 146 - protein, 8 aa, synthetic construct
  REGION 1..8: note = Synthetic
GESMTQGY

SEQ ID NO: 147 - protein, 8 aa, synthetic construct
  REGION 1..8: note = Synthetic
GDSMTQGY

SEQ ID NO: 148 - protein, 117 aa, synthetic construct
  REGION 1..117: note = Synthetic
QVKLQESGPELVKPGASVKISCKASGYSFTDYNMNWVKQSKGKSLEWIGIIHPNSGTTTYNQKFKGKATLTVDQSSSTAYLQLNSLTSEDSAVYYCARSKLRFFDYWGQGTTVTVSS

SEQ ID NO: 149 - protein, 107 aa, synthetic construct
  REGION 1..107: note = Synthetic
DIKLTQSPSSMYASLGERVTITCKASQDIYSYLSWFQQKPGKSPKTLIYRANRLIDGVPSRFSGSGSGQDYSLTISSLEYEHMGIYYCLQYDEFPFTFGSGTKLEIK

SEQ ID NO: 150 - protein, 107 aa, synthetic construct
  REGION 1..107: note = Synthetic
DIQMTQSPSSLSASVGDRVTITCQASQDISNYLNWYQQKPGKAPKLLIYDASNLETGVPSRFSGSGSGTDFTFTISSLQPEDIATYYCQQYDNLPCSFGQGTKLEIK

SEQ ID NO: 151 - protein, 118 aa, synthetic construct
  REGION 1..118: note = Synthetic
  REGION 99..103: note = misc_feature - X can be any naturally occurring amino acid
QVQLVQSGSELKKPGASVKVSCKASGYTFTSYAMNWVRQAPGQGLEWMGWINTNTGNPTYAQGFTGRFVFSLDTSVSTAYLQISSLKAEDTAVYYCARXXXXXYFDYWGQGTLVTVSS

SEQ ID NO: 152 - protein, 118 aa, synthetic construct
  REGION 1..118: note = Synthetic
  REGION 99..103: note = misc_feature - X can be any naturally occurring amino acid
QVQLVQSGAEVKKPGASVKVSCKASGYTFTSYYMHWVRQAPGQGLEWMGIINPSGGSTSYAQKFQGRVTMTRDTSTSTVYMELSSLRSEDTAVYYCARXXXXXYFDYWGQGTLVTVSS

SEQ ID NO: 153 - protein, 107 aa, synthetic construct
  REGION 1..107: note = Synthetic
DIQLTQSPSSLSASVGDRVTITCKASQDIYSYLSWFQQKPGKAPKTLIYRANRLIDGVPSRFSGSGSGQDYTFTISSLQPEDIATYYCLQYDEFPFTFGQGTKLEIK

SEQ ID NO: 154 - protein, 117 aa, synthetic construct
  REGION 1..117: note = Synthetic
QVQLVQSGSELKKPGASVKVSCKASGYSFTDYNMNWVRQAPGQGLEWIGIIHPNSGTTTYNQKFKGRAVLSVDQSVSTAYLQISSLKAEDTAVYYCARSKLRFFDYWGQGTLVTVSS

SEQ ID NO: 155 - protein, 117 aa, synthetic construct
  REGION 1..117: note = Synthetic
QVQLVQSGAEVKKPGASVKVSCKASGYSFTDYNMNWVRQAPGQGLEWIGIIHPNSGTTTYNQKFKGRATLTVDQSTSTAYMELSSLRSEDTAVYYCARSKLRFFDYWGQGTLVTVSS

SEQ ID NO: 156-157 - skipped (2 entries)

SEQ ID NO: 158 - protein, 20 aa, synthetic construct
  REGION 1..20: note = Synthetic
  REGION 3..4: note = misc_feature - X can be any naturally occurring amino acid
  REGION 13..14: note = misc_feature - X can be any naturally occurring amino acid
TDXXRQFQADFTXXSDQEPL

SEQ ID NO: 159 - protein, 11 aa, synthetic construct
  REGION 1..11: note = Artificial Sequence
TTGGETRQQIQ

SEQ ID NO: 160 - skipped

SEQ ID NO: 161 - protein, 22 aa, synthetic construct
  REGION 1..22: note = Artificial Sequence
  REGION 4..6: note = misc_feature - X can be any naturally occurring amino acid
TDMXXXFQADFTSLSNQEPLHV

SEQ ID NO: 162 - protein, 402 aa, cynomolgus
MQMSPALACLVLGLAFVFGEGSTVHHPPSYVAHLASDFGVRVFQQVAQASKDRNVVFSPYGVASVLAMLQLTTGGETRQQIQAAMGFKIDDKGMAPALRHLYKELLGPWNKDEISTTDAIFVQRDLKLVQGFMPHFFRLFRSTVKQVDFSEAERARFIINDWVKTHTKGMISDLLGKGAVDQLTRLVLVNALYFNGHWKTPFPDSSTHRRLFHKSDGSTVSVPMMAQTNKFNYTEFTTPDGHYYDILELPYHGNTLSMFIAAPYEKQVPLSALTNILSAQLISHWKGNMTRLPRLLVLPKFSLETEVDLRKPLENLGMTDMFRQFQADFTSLSNQEPLHVAQALQKVKIEVNESGTVASSSTAVIVSARMAPEEIIMDRPFLFVVRHNPTGTVLFMGQVMEP

SEQ ID NO: 163 - protein, 402 aa, Mus musculus
MQMSSALACLILGLVLVSGKGFTLPLRESHTAHQATDFGVKVFQQVVQASKDRNVVFSPYGVSSVLAMLQMTTAGKTRRQIQDAMGFKVNEKGTAHALRQLSKELMGPWNKNEISTADAIFVQRDLELVQGFMPHFFKLFQTMVKQVDFSEVERARFIINDWVERHTKGMISDLLAKGAVDELTRLVLVNALYFSGQWKTPFLEASTHQRLFHKSDGSTVSVPMMAQSNKFNYTEFTTPDGLEYDVVELPYQGDTLSMFIAAPFEKDVHLSALTNILDAELIRQWKGNMTRLPRLLILPKFSLETEVDLRGPLEKLGMPDMFSATLADFTSLSDQEQLSVAQALQKVRIEVNESGTVASSSTAFVISARMAPTEMVIDRSFLFVVRHNPTETILFMGQVMEP

SEQ ID NO: 164 - protein, 402 aa, Rattus norvegicus
MQMSSALTCLTLGLVLVFGKGFASPLPESHTAQQATNFGVKVFQHVVQASKDRNVVFSPYGVSSVLAMLQLTTAGKTRQQIQDAMGFNISERGTAPALRKLSKELMGSWNKNEISTADAIFVQRDLELVQGFMPHFFKLFRTTVKQVDFSEVERARFIINDWVERHTKGMISDLLAKGAVNELTRLVLVNALYFNGQWKTPFLEASTHQRLFHKSDGSTISVPMMAQNNKFNYTEFTTPDGHEYDILELPYHGETLSMFIAAPFEKDVPLSAITNILDAELIRQWKSNMTRLPRLLILPKFSLETEVDLRGPLEKLGMTDIFSSTQADFTSLSDQEQLSVAQALQKVKIEVNESGTVASSSTAILVSARMAPTEMVLDRSFLFVVRHNPTETILFMGQLMEP

SEQ ID NO: 165 - protein, 6 aa, synthetic construct
  REGION 1..6: note = Synthetic
QDIYSY

SEQ ID NO: 166 - protein, 9 aa, synthetic construct
  REGION 1..9: note = Synthetic
LQYDEFPFT

SEQ ID NO: 167 - skipped

SEQ ID NO: 168 - protein, 8 aa, synthetic construct
  REGION 1..8: note = Synthetic
GYSFTDYN

SEQ ID NO: 169 - protein, 9 aa, synthetic construct
  REGION 1..9: note = Synthetic
LQYDEFPFT

SEQ ID NO: 170 - skipped